European Patent Application EP 4 623 928 A1, published October 1, 2025. Title: GLP-1R ANTAGONISTS FOR THE TREATMENT OF CANCER. Applicant: Paolo Fiorina. Application EP. The sequence listing filed with the application follows.

SEQUENCE LISTING (4 sequences)

SEQ ID NO: 1 - DNA, 21 bp, synthetic construct
  source 1..21: mol_type = other DNA
tgctatcggcgtcaactttct

SEQ ID NO: 2 - DNA, 20 bp, synthetic construct
  source 1..20: mol_type = other DNA
attcaagtgctccagcctcc

SEQ ID NO: 3 - DNA, 30 bp, synthetic construct
  source 1..30: mol_type = other DNA
ccagggctgccatttgcagtggcaaagtgg

SEQ ID NO: 4 - DNA, 30 bp, synthetic construct
  source 1..30: mol_type = other DNA
cctggaagatggtgatgggvttcccgttga